European Patent Application EP 4 786 492 A1, published August 5, 2026. Title: 特异性识别Delta样配体3的单克隆抗体及其应用. Applicant: 海南先声再明医药股份有限公司. The sequence listing filed with the application follows.

SEQUENCE LISTING (378 sequences)

SEQ ID NO: 1 - protein, 118 aa, synthetic construct
QVQLVQSGAEVKKPGASVKVSCKASGYTFTNYGMNWVRQAPGQGLEWMGWINTYTGEPTYADDFKGRVTMTTDTSTSTAYMELRSLRSDDTAVYYCARIGDSSPSDYWGQGTLVTVSS

SEQ ID NO: 2 - protein, 107 aa, synthetic construct
EIVMTQSPATLSVSPGERATLSCKASQSVSNDVVWYQQKPGQAPRLLIYYASNRYTGIPARFSGSGSGTEFTLTISSLQSEDFAVYYCQQDYTSPWTFGQGTKLEIK

SEQ ID NO: 3 - protein, 448 aa, synthetic construct
QVQLVQSGAEVKKPGASVKVSCKASGYTFTNYGMNWVRQAPGQGLEWMGWINTYTGEPTYADDFKGRVTMTTDTSTSTAYMELRSLRSDDTAVYYCARIGDSSPSDYWGQGTLVTVSSASTKGPSVFPLAPSSKSTSGGTAALGCLVKDYFPEPVTVSWNSGALTSGVHTFPAVLQSSGLYSLSSVVTVPSSSLGTQTYICNVNHKPSNTKVDKKVEPKSCDKTHTCPPCPAPELLGGPSVFLFPPKPKDTLMISRTPEVTCVVVDVSHEDPEVKFNWYVDGVEVHNAKTKPREEQYNSTYRVVSVLTVLHQDWLNGKEYKCKVSNKALPAPIEKTISKAKGQPREPQVYTLPPSREEMTKNQVSLTCLVKGFYPSDIAVEWESNGQPENNYKTTPPVLDSDGSFFLYSKLTVDKSRWQQGNVFSCSVMHEALHNHYTQKSLSLSPGK

SEQ ID NO: 4 - protein, 214 aa, synthetic construct
EIVMTQSPATLSVSPGERATLSCKASQSVSNDVVWYQQKPGQAPRLLIYYASNRYTGIPARFSGSGSGTEFTLTISSLQSEDFAVYYCQQDYTSPWTFGQGTKLEIKRTVAAPSVFIFPPSDEQLKSGTASVVCLLNNFYPREAKVQWKVDNALQSGNSQESVTEQDSKDSTYSLSSTLTLSKADYEKHKVYACEVTHQGLSSPVTKSFNRGEC

SEQ ID NO: 5 - protein, 241 aa, synthetic construct
QVQLQESGPGLVKPSETLSLTCTVSGGSISSYYWSWIRQPPGKCLEWIGYVYYSGTTNYNPSLKSRVTISVDTSKNQFSLKLSSVTAADTAVYYCASIAVTGFYFDYWGQGTLVTVSSGGGGSGGGGSGGGGSEIVLTQSPGTLSLSPGERVTLSCRASQRVNNNYLAWYQQRPGQAPRLLIYGASSRATGIPDRFSGSGSGTDFTLTISRLEPEDFAVYYCQQYDRSPLTFGCGTKLEIK

SEQ ID NO: 6 - protein, 473 aa, synthetic construct
QVQLQESGPGLVKPSETLSLTCTVSGGSISSYYWSWIRQPPGKCLEWIGYVYYSGTTNYNPSLKSRVTISVDTSKNQFSLKLSSVTAADTAVYYCASIAVTGFYFDYWGQGTLVTVSSGGGGSGGGGSGGGGSEIVLTQSPGTLSLSPGERVTLSCRASQRVNNNYLAWYQQRPGQAPRLLIYGASSRATGIPDRFSGSGSGTDFTLTISRLEPEDFAVYYCQQYDRSPLTFGCGTKLEIKEPKSSDKTHTCPPCPAPELLGGPSVFLFPPKPKDTLMISRTPEVTCVVVDVSHEDPEVKFNWYVDGVEVHNAKTKPREEQYNSTYRVVSVLTVLHQDWLNGKEYKCKVSNKALPAPIEKTISKAKGQPREPQVYTLPPSREEMTKNQVSLTCLVKGFYPSDIAVEWESNGQPENNYKTTPPVLDSDGSFFLYSKLTVDKSRWQQGNVFSCSVMHEALHNHYTQKSLSLSPGK

SEQ ID NO: 7 - protein, 248 aa, synthetic construct
QLQLQESGPGLVKPSETLSLTCTVSGGSISSSSYYWGWIRQPPGKGLEWIGSIYYSGNIYHNPSLKSRVSISVDTSKNQFSLRLSSVTAADTAVYYCAREIIVGATHFDYWGQGTLVTVSSGGGGSGGGGSGGGGSGGGGSAIQMTQSPSSLSASVGDRVTITCRASQGIRNDLGWYQQKPGKAPELLIYAASSLQSGVPSRFSGSGSGTDFTLTISSLQPEDFATYYCLQDYNYPLTFGPGTKVDIK

SEQ ID NO: 8 - protein, 480 aa, synthetic construct
QLQLQESGPGLVKPSETLSLTCTVSGGSISSSSYYWGWIRQPPGKGLEWIGSIYYSGNIYHNPSLKSRVSISVDTSKNQFSLRLSSVTAADTAVYYCAREIIVGATHFDYWGQGTLVTVSSGGGGSGGGGSGGGGSGGGGSAIQMTQSPSSLSASVGDRVTITCRASQGIRNDLGWYQQKPGKAPELLIYAASSLQSGVPSRFSGSGSGTDFTLTISSLQPEDFATYYCLQDYNYPLTFGPGTKVDIKEPKSADKTHTCPPCPAPELLGGPSVFLFPPKPKDTLMISRTPEVTCVVVDVSHEDPEVKFNWYVDGVEVHNAKTKPREEQYNSTYRVVSVLTVLHQDWLNGKEYKCKVSNKALPAPIEKTISKAKGQPREPQVYTLPPSREEMTKNQVSLTCLVKGFYPSDIAVEWESNGQPENNYKTTPPVLDSDGSFFLYSKLTVDKSRWQQGNVFSCSVMHEALHNHYTQKSLSLSPGK

SEQ ID NO: 9 - protein, 124 aa, synthetic construct
QVQLVQSGAEVKKPGASVKVSCKASGYTFTSYYVHWVRQAPGQGLEWMVIINPGGGTTSYAQKFLGRVTMTRDTSTNTVYMELKSLRSEDTAVYYCARGEAVTGNYFYYGMDVWGQGTTVTVSS

SEQ ID NO: 10 - protein, 107 aa, synthetic construct
DIQMTQSPSAMSASVGDRVTITCRASQGISNYLVWFQQKPGKAPKRLIYAVSSLYSGVPSRFSGSGSGTEFTLTISSLQPEDFATYYCLQHDSYPYTFGQGTKLEIK

SEQ ID NO: 11 - protein, 454 aa, synthetic construct
QVQLVQSGAEVKKPGASVKVSCKASGYTFTSYYVHWVRQAPGQGLEWMVIINPGGGTTSYAQKFLGRVTMTRDTSTNTVYMELKSLRSEDTAVYYCARGEAVTGNYFYYGMDVWGQGTTVTVSSASTKGPSVFPLAPSSKSTSGGTAALGCLVKDYFPEPVTVSWNSGALTSGVHTFPAVLQSSGLYSLSSVVTVPSSSLGTQTYICNVNHKPSNTKVDKKVEPKSCDKTHTCPPCPAPELLGGPSVFLFPPKPKDTLMISRTPEVTCVVVDVSHEDPEVKFNWYVDGVEVHNAKTKPREEQYNSTYRVVSVLTVLHQDWLNGKEYKCKVSNKALPAPIEKTISKAKGQPREPQVYTLPPSREEMTKNQVSLTCLVKGFYPSDIAVEWESNGQPENNYKTTPPVLDSDGSFFLYSKLTVDKSRWQQGNVFSCSVMHEALHNHYTQKSLSLSPGK

SEQ ID NO: 12 - protein, 214 aa, synthetic construct
DIQMTQSPSAMSASVGDRVTITCRASQGISNYLVWFQQKPGKAPKRLIYAVSSLYSGVPSRFSGSGSGTEFTLTISSLQPEDFATYYCLQHDSYPYTFGQGTKLEIKRTVAAPSVFIFPPSDEQLKSGTASVVCLLNNFYPREAKVQWKVDNALQSGNSQESVTEQDSKDSTYSLSSTLTLSKADYEKHKVYACEVTHQGLSSPVTKSFNRGEC

SEQ ID NO: 13 - protein, 466 aa, synthetic construct
AGVFELQIHSFGPGPGPGAPRSPCSARLPCRLFFRVCLKPGLSEEAAESPCALGAALSARGPVYTEQPGAPAPDLPLPDGLLQVPFRDAWPGTFSFIIETWREELGDQIGGPAWSLLARVAGRRRLAAGGPWARDIQRAGAWELRFSYRARCEPPAVGTACTRLCRPRSAPSRCGPGLRPCAPLEDECEAPLVCRAGCSPEHGFCEQPGECRCLEGWTGPLCTVPVSTSSCLSPRGPSSATTGCLVPGPGPCDGNPCANGGSCSETPRSFECTCPRGFYGLRCEVSGVTCADGPCFNGGLCVGGADPDSAYICHCPPGFQGSNCEKRVDRCSLQPCRNGGLCLDLGHALRCRCRAGFAGPRCEHDLDDCAGRACANGGTCVEGGGAHRCSCALGFGGRDCRERADPCAARPCAHGGRCYAHFSGLVCACAPGYMGARCEFPVHPDGASALPAAPPGLRPGDPQRYL

SEQ ID NO: 14 - protein, 464 aa, synthetic construct
AGVFELQIHSFGPGPGPGAPRSPCSARGPCRLFFRVCLKPGLSEEAAESPCALGAALSARGPVYTEQPEAPAPDLPLPNGLLQVPFRDAWPGTFSLIIETWREELGDQIGGPAWSLLARVTRRRRLAAGGPWARDIQRAGAWELRFSYRARCELPAVGTACTRLCRPRSAPSRCGPGLRPCAPLEDECEAPPVCRAGCSLEHGFCEQPGECRCLEGWTGPLCMVPVSTSSCLGLRGPSSTTTGCLVPGPGPCDGNPCANGGSCSETPGSFECTCPRGFYGLRCEVSGVTCADGPCFNGGLCVGGADPDSAYICHCPPGFQGSNCEKRVDRCSLQPCRNGGLCLDLGHALRCRCRAGFAGPRCEHDLDDCAGRACANGGTCVEGGGAHRCSCALGFGGRNCRERADPCAARPCAHGGRCYAHFSGLVCACAPGYMGARCEFPVHPDGVSALPAAPPGLRPGDPQR

SEQ ID NO: 15 - protein, 49 aa, synthetic construct
AGVIAVIVVVVIAIVAGIVVLVISRKKRMAKYEKAEIKEMGEMHRELNA

SEQ ID NO: 16 - protein, 458 aa, synthetic construct
HSFGPGPGLGTPRSPCNARGPCRLFFRVCLKPGVSQEATESLCALGAALSTSVPVYTEHPGESAAALPLPDGLVRVPFRDAWPGTFSLVIETWREQLGEHAGGPAWNLLARVVGRRRLAAGGPWARDVQRTGTWELHFSYRARCEPPAVGAACARLCRSRSAPSRCGPGLRPCTPFPDECEAPSVCRPGCSPEHGYCEEPDECRCLEGWTGPLCTVPVSTSSCLNSRVPGPASTGCLLPGPGPCDGNPCANGGSCSETSGSFECACPRGFYGLRCEVSGVTCADGPCFNGGLCVGGEDPDSAYVCHCPPGFQGSNCEKRVDRCSLQPCQNGGLCLDLGHALRCRCRAGFAGPRCEHDLDDCAGRACANGGTCVEGGGSRRCSCALGFGGRDCRERADPCASRPCAHGGRCYAHFSGLVCACAPGYMGVRCEFAVRPDGADAVPAAPRGLRQADPQRFL

SEQ ID NO: 17 - protein, 232 aa, synthetic construct
EPKSSDKTHTCPPCPAPELLGGPSVFLFPPKPKDTLMISRTPEVTCVVVDVSHEDPEVKFNWYVDGVEVHNAKTKPREEQYNSTYRVVSVLTVLHQDWLNGKEYKCKVSNKALPAPIEKTISKAKGQPREPQVYTLPPSREEMTKNQVSLTCLVKGFYPSDIAVEWESNGQPENNYKTTPPVLDSDGSFFLYSKLTVDKSRWQQGNVFSCSVMHEALHNHYTQKSLSLSPGK

SEQ ID NO: 18 - protein, 118 aa, synthetic construct
QIQLVQSGPELKKPGETVKISCKASGYTFTTYGMSWVKQAPGKGLKWMGWINTYSGVPTYADDFKGRFAFSLETSASTAYLQINNLKNEDTATYFCARIGDYDYGEYWGQGTLVTVSA

SEQ ID NO: 19 - protein, 112 aa, synthetic construct
DVVMTQTPLTLAVTTGQPASISCKSSQSLLDSDGKTYLNWLLQRPGQSPKRLLYLVSQLDSGVPDRFSGSGSGTDFTLKISRVEAEDLGVYYCWQGTHFPYTFGGGTKLEIK

SEQ ID NO: 20 - protein, 121 aa, synthetic construct
QIQLVQSGPELKKPGETVKISCKASGYTFTNYGMNWLKQAPGKGLKWMGWINTYTGESTYADDFKGRFAFSLETSASTVYLQINNLKNEDMATYFCARMGDGYYDFTMDYWGQGTSVTVSS

SEQ ID NO: 21 - protein, 106 aa, synthetic construct
QIVLTQSPAIMSASPGEKVTMTCSARSSVSYMQWYQQKSGTSPKRWIYDTSKLASGVPARFSGSGSGTSYSLTISTMEAEDAATYYCQQWSSDPPTFGGGTKLEIK

SEQ ID NO: 22 - protein, 119 aa, synthetic construct
QVQLQQSGTELMKPGASVKLSCKATGYTFTGNWIEWVKQRPGHGLEWIGEILPGTGSTQYNEKFKGKATFTADPSSNTAYMQLSSLTTEDSAIYYCARWGSTVVAYDYWGQGTTLTVSS

SEQ ID NO: 23 - protein, 107 aa, synthetic construct
DVQITQSPSYLAASPGETITINCRASKSISKYLAWYQEKPGKTNKLLIYSGSTLHSGIPSRFSGSGSGTDFTLTISSLEPEDFAIYYCQQHNEYPLTFGGGTKLELK

SEQ ID NO: 24 - protein, 117 aa, synthetic construct
QVQLQQPGAELVKPGASVKLSCKASGYTFTSYWINWVKQRPGQGLEWIGNIYPGSSSPNYNEKFKSKATLTVDTSSSTAYMQLSSLTSDDSAVYYCARSLLYAMDYWGQGTSVTVSS

SEQ ID NO: 25 - protein, 111 aa, synthetic construct
DIVLTQSPASLAVSLGQRATISCRASESVDYDGDSYMNWYQQKPGQPPKLLIYVASNLESGIPARFSGSGSGTDFILNIHPVEEEDAATYYCLQSNEAPYTFGSGTKLEIK

SEQ ID NO: 26 - protein, 117 aa, synthetic construct
QVQLQQSGAELMKPGASVTLSCKATGYTLPGYWIEWVKQRPGHGLEWIGEILPGSSSANYNEKFKGKATFTADTSSNTAYMQLSSLTTEDSAIYYCASTYGTSLDYWGQGTTLTVSS

SEQ ID NO: 27 - protein, 107 aa, synthetic construct
DIVLTQSPATLSVTPGDSVSLSCRASQSVSNDLHWYQQKSHESPRLLIKYASQSISGIPSRFSGSGSGTDFTLTINSVETEDFGMYFCQQSNNWPYTFGGGTKLEMK

SEQ ID NO: 28 - protein, 119 aa, synthetic construct
QVQLQQPGAELVRPGTSVKLSCKASGYTFTSYWMHWVRQRPGQGLEWIGVIDPSDSLANYNQEFKGKATLTVDTSSSTAYMQLSSLTSEDSAVYYCARDSTVVAPMDYWGQGTSVTVSS

SEQ ID NO: 29 - protein, 107 aa, synthetic construct
DVQITQSPSYLAASPGETITINCRATKSISKYLAWYQEKPGKTNKLLIFSGSTLQSGIPSRFRGSGSGTDFTLTISSLEPEDFAMYYCQQHHEYPYTFGGGTKLEIK

SEQ ID NO: 30 - protein, 119 aa, synthetic construct
QVQLQQPGAELVRPGTSVKLSCKASGYTFTSYWMHWVKQRPGQGLEWIGVIDPSDSLANYNQEFKGKATLTVDTSSSTAYMQLSSLTSEDSAVYYCARDSTVVAPMDYWGQGTSVTVSS

SEQ ID NO: 31 - protein, 107 aa, synthetic construct
DVQITQSPSYLAASPGETITINCRASTSISKYLAWYQERPGKTNKLLIYSGSTLQSGIPSRFRGSGSGTDFTLTISSLEPEDFAMYYCQQHHVYPYTFGGGTKLEIK

SEQ ID NO: 32 - protein, 122 aa, synthetic construct
EVQLQQSGPVLVKPGASVKMSCKASGYTFTDYYMNWVKRSHGKSLEWIGIINPYNGGTSYNQKFRGKATLTVDKSSNTAYMELNSLTSEDSAVYYCSRYDYDYDVEGAMDYWGQGTSVTVSS

SEQ ID NO: 33 - protein, 107 aa, synthetic construct
DIVMTQSQKFMSTSVGDRVSITCKASQNVGTAVAWYQQKPGQSPKLLIFSASIRYTGVPDRFTGSGSGTDFTLTISNMQSEDLADYFCQQYSSSPYTFGGGTKLEIK

SEQ ID NO: 34 - protein, 118 aa, synthetic construct
EVQLQQSGTVLARPGASVKMSCKTSGYTFTSYWMHWVKQSPGQGLEWIGTIYPGNSDTRYNQKFKDKAYVTAVTSASTAYMELSSLTNEESAVYYCTRSYDYGDLDYWGQGTTLTVSS

SEQ ID NO: 35 - protein, 107 aa, synthetic construct
DIVMTQSPATLSVTPGDRVSLSCRASQTISDYLHWYQQRSHESPRLLIKYASQSISGIPSRFSGSGSGSDFTLSINSVEPEDVGVYYCQNGHSFPLTFGAGTKLELK

SEQ ID NO: 36 - protein, 120 aa, synthetic construct
QVQLQQSGAELARPGASMKLSCKASGYTFTSYGISWVKQITGQGLEWIGEIFPRSGNTYDNENFRGKATLTADKSSSTAYLEVRSLTSEDSAVYFCARTTVFAPYYFDYWGQGTTLTVSS

SEQ ID NO: 37 - protein, 107 aa, synthetic construct
DIQMTQSPASLSVSVGETVTITCRASENINSNLAWYQQKQGKSPQLLVYAATNLADGVPSRFSGSGSGTQFSLKISGLQSEDFGSYYCQHFWGLPWTFGGGTKLEIR

SEQ ID NO: 38 - protein, 124 aa, synthetic construct
EVQLQQSGPELVKPGASVKISCKASGYTFTDYYMNWVKQSHGKSLEWIGDISPNYGGTNYNQKFKGKATLTVDKSSSTACMELRSLTSEDSAVYYCTRSFYYYGTGYDWYFDVWGTGTTVTVSS

SEQ ID NO: 39 - protein, 107 aa, synthetic construct
DIVLTQSPATLSVTPGDSVSLSCRASQSISNNLHWYQQKSHESPRLLIKYASQSISGIPSRFSGSGSGTDFTLSINSVETEDFGMYFCQQSNSWPWTFGGGTKLEIK

SEQ ID NO: 40 - protein, 122 aa, synthetic construct
QVQLQQSGPELVKPGASVKISCKASGYTFTDYYIHWVKQRPGQGLEWIGWTLPGSGSPYYNEKFKGKATLTVDKSSSTAYMLLSSLTSEDSAVYFCARWHYYYGSSYHFDYWGQGTTLTVSS

SEQ ID NO: 41 - protein, 112 aa, synthetic construct
DVLMTQTPLSLPVSLGDQASISCRSSQSIVHSDGNTYLEWYLQKPGQSPKLLIYKVSNRFSGVPDRFSGSGSGTDFTLKISRVEAEDLGFYYCFQGSHVPFTFGSGTKLEIK

SEQ ID NO: 42 - protein, 119 aa, synthetic construct
QVQLQQSGAELVKPGASVRISCKASGYAFSNYWINWVKQRPGKGLEWIGQINPGDGDTIYNGKFKGKATLTADKSSSTAYMQLSSLTSEDSAVYFCEREGRNYGDFAYWGQGTTLTVSS

SEQ ID NO: 43 - protein, 111 aa, synthetic construct
DIVLTQSPASLAVSLGQRATISCRASKSVSTSGFSYMHWYQQKPGQPPKLLIYLASNLESGVPARFSGSGSGTDFTLNIHPVEEEDAATYYCQHSRELPFTFGSGTKLEIK

SEQ ID NO: 44 - protein, 124 aa, synthetic construct
EVQLHQSGPELVKPGTSVKISCKASGYTFTDYYMNWVKQSHGKSLEWIGDINPNHGDTGYNQKFTGKATLTVDKSSSTAYMELRSLTSEDSAVYYCARNFFYYGTTYGWYFDVWGTGTTVTVSS

SEQ ID NO: 45 - protein, 107 aa, synthetic construct
DIQMTQSSSSFSVSLGDRVTITCKASEDIYNRLAWYQQKPGNTPRLLISGATSLETGVPSRFSGSGSGKDFTLSITSLQTEDVATYYCQQYWSLPWTFGGGTKLEIK

SEQ ID NO: 46 - protein, 117 aa, synthetic construct
EVKLEESGGGLVQPGGSMKLSCVASGITFSNFWMNWVRQSPEKGLEWVAQIRLKSDDYATHYAESVKGRFTISRDDSKGSVYLQMNNLRTEDTGIHYCTTGYYFDYWGQGTTLTVSS

SEQ ID NO: 47 - protein, 107 aa, synthetic construct
NIVMTQSPKSMSMSVGERVTLSCKASENVGTYVSWFQQKPEQSPKLLIYGASNRYTGVPDRFTGSGSATDFTLTISSVQAEDLADYHCGQFYSFPCTFGGGTKLEIK

SEQ ID NO: 48 - protein, 119 aa, synthetic construct
EVNLEESGGGLVQPGGSMKLSCVASGFAFSNFWMQWVRQSPEKGLEWVAQIRLKSDNYAAHYAESVKGRFTISRDDSKSSVYLQLNNLRAEDTGTYYCTQGNWVGFAYWGQGTLVTVSA

SEQ ID NO: 49 - protein, 107 aa, synthetic construct
DIVMTQSQKFMSTTIGDRVSITCKASQNVGTTVAWYQQKPGQSPNLLLYSTSNRFTGVPDRFTGSGSGTDFTLTITNMQSEDLADYFCQQYNNYPLTFGGGTKLEIK

SEQ ID NO: 50 - protein, 5 aa, synthetic construct
TYGMS

SEQ ID NO: 51 - protein, 17 aa, synthetic construct
WINTYSGVPTYADDFKG

SEQ ID NO: 52 - protein, 9 aa, synthetic construct
IGDYDYGEY

SEQ ID NO: 53 - protein, 16 aa, synthetic construct
KSSQSLLDSDGKTYLN

SEQ ID NO: 54 - protein, 7 aa, synthetic construct
LVSQLDS

SEQ ID NO: 55 - protein, 9 aa, synthetic construct
WQGTHFPYT

SEQ ID NO: 56 - protein, 5 aa, synthetic construct
NYGMN

SEQ ID NO: 57 - protein, 17 aa, synthetic construct
WINTYTGESTYADDFKG

SEQ ID NO: 58 - protein, 12 aa, synthetic construct
MGDGYYDFTMDY

SEQ ID NO: 59 - protein, 10 aa, synthetic construct
SARSSVSYMQ

SEQ ID NO: 60 - protein, 7 aa, synthetic construct
DTSKLAS

SEQ ID NO: 61 - protein, 9 aa, synthetic construct
QQWSSDPPT

SEQ ID NO: 62 - protein, 5 aa, synthetic construct
GNWIE

SEQ ID NO: 63 - protein, 17 aa, synthetic construct
EILPGTGSTQYNEKFKG

SEQ ID NO: 64 - protein, 10 aa, synthetic construct
WGSTVVAYDY

SEQ ID NO: 65 - protein, 11 aa, synthetic construct
RASKSISKYLA

SEQ ID NO: 66 - protein, 7 aa, synthetic construct
SGSTLHS

SEQ ID NO: 67 - protein, 9 aa, synthetic construct
QQHNEYPLT

SEQ ID NO: 68 - protein, 5 aa, synthetic construct
SYWIN

SEQ ID NO: 69 - protein, 17 aa, synthetic construct
NIYPGSSSPNYNEKFKS

SEQ ID NO: 70 - protein, 8 aa, synthetic construct
SLLYAMDY

SEQ ID NO: 71 - protein, 15 aa, synthetic construct
RASESVDYDGDSYMN

SEQ ID NO: 72 - protein, 7 aa, synthetic construct
VASNLES

SEQ ID NO: 73 - protein, 9 aa, synthetic construct
LQSNEAPYT

SEQ ID NO: 74 - protein, 5 aa, synthetic construct
GYWIE

SEQ ID NO: 75 - protein, 17 aa, synthetic construct
EILPGSSSANYNEKFKG

SEQ ID NO: 76 - protein, 8 aa, synthetic construct
TYGTSLDY

SEQ ID NO: 77 - protein, 11 aa, synthetic construct
RASQSVSNDLH

SEQ ID NO: 78 - protein, 7 aa, synthetic construct
YASQSIS

SEQ ID NO: 79 - protein, 9 aa, synthetic construct
QQSNNWPYT

SEQ ID NO: 80 - protein, 5 aa, synthetic construct
SYWMH

SEQ ID NO: 81 - protein, 17 aa, synthetic construct
VIDPSDSLANYNQEFKG

SEQ ID NO: 82 - protein, 10 aa, synthetic construct
DSTVVAPMDY

SEQ ID NO: 83 - protein, 11 aa, synthetic construct
RATKSISKYLA

SEQ ID NO: 84 - protein, 7 aa, synthetic construct
SGSTLQS

SEQ ID NO: 85 - protein, 9 aa, synthetic construct
QQHHEYPYT

SEQ ID NO: 86 - protein, 5 aa, synthetic construct
SYWMH

SEQ ID NO: 87 - protein, 17 aa, synthetic construct
VIDPSDSLANYNQEFKG

SEQ ID NO: 88 - protein, 10 aa, synthetic construct
DSTVVAPMDY

SEQ ID NO: 89 - protein, 11 aa, synthetic construct
RASTSISKYLA

SEQ ID NO: 90 - protein, 7 aa, synthetic construct
SGSTLQS

SEQ ID NO: 91 - protein, 9 aa, synthetic construct
QQHHVYPYT

SEQ ID NO: 92 - protein, 5 aa, synthetic construct
DYYMN

SEQ ID NO: 93 - protein, 17 aa, synthetic construct
IINPYNGGTSYNQKFRG

SEQ ID NO: 94 - protein, 13 aa, synthetic construct
YDYDYDVEGAMDY

SEQ ID NO: 95 - protein, 11 aa, synthetic construct
KASQNVGTAVA

SEQ ID NO: 96 - protein, 7 aa, synthetic construct
SASIRYT

SEQ ID NO: 97 - protein, 9 aa, synthetic construct
QQYSSSPYT

SEQ ID NO: 98 - protein, 5 aa, synthetic construct
SYWMH

SEQ ID NO: 99 - protein, 17 aa, synthetic construct
TIYPGNSDTRYNQKFKD

SEQ ID NO: 100 - protein, 9 aa, synthetic construct
SYDYGDLDY

SEQ ID NO: 101 - protein, 11 aa, synthetic construct
RASQTISDYLH

SEQ ID NO: 102 - protein, 7 aa, synthetic construct
YASQSIS

SEQ ID NO: 103 - protein, 9 aa, synthetic construct
QNGHSFPLT

SEQ ID NO: 104 - protein, 5 aa, synthetic construct
SYGIS

SEQ ID NO: 105 - protein, 17 aa, synthetic construct
EIFPRSGNTYDNENFRG

SEQ ID NO: 106 - protein, 11 aa, synthetic construct
TTVFAPYYFDY

SEQ ID NO: 107 - protein, 11 aa, synthetic construct
RASENINSNLA

SEQ ID NO: 108 - protein, 7 aa, synthetic construct
AATNLAD

SEQ ID NO: 109 - protein, 9 aa, synthetic construct
QHFWGLPWT

SEQ ID NO: 110 - protein, 5 aa, synthetic construct
DYYMN

SEQ ID NO: 111 - protein, 17 aa, synthetic construct
DISPNYGGTNYNQKFKG

SEQ ID NO: 112 - protein, 15 aa, synthetic construct
SFYYYGTGYDWYFDV

SEQ ID NO: 113 - protein, 11 aa, synthetic construct
RASQSISNNLH

SEQ ID NO: 114 - protein, 7 aa, synthetic construct
YASQSIS

SEQ ID NO: 115 - protein, 9 aa, synthetic construct
QQSNSWPWT

SEQ ID NO: 116 - protein, 5 aa, synthetic construct
DYYIH

SEQ ID NO: 117 - protein, 17 aa, synthetic construct
WTLPGSGSPYYNEKFKG

SEQ ID NO: 118 - protein, 13 aa, synthetic construct
WHYYYGSSYHFDY

SEQ ID NO: 119 - protein, 16 aa, synthetic construct
RSSQSIVHSDGNTYLE

SEQ ID NO: 120 - protein, 7 aa, synthetic construct
KVSNRFS

SEQ ID NO: 121 - protein, 9 aa, synthetic construct
FQGSHVPFT

SEQ ID NO: 122 - protein, 5 aa, synthetic construct
NYWIN

SEQ ID NO: 123 - protein, 17 aa, synthetic construct
QINPGDGDTIYNGKFKG

SEQ ID NO: 124 - protein, 10 aa, synthetic construct
EGRNYGDFAY

SEQ ID NO: 125 - protein, 15 aa, synthetic construct
RASKSVSTSGFSYMH

SEQ ID NO: 126 - protein, 7 aa, synthetic construct
LASNLES

SEQ ID NO: 127 - protein, 9 aa, synthetic construct
QHSRELPFT

SEQ ID NO: 128 - protein, 5 aa, synthetic construct
DYYMN

SEQ ID NO: 129 - protein, 17 aa, synthetic construct
DINPNHGDTGYNQKFTG

SEQ ID NO: 130 - protein, 15 aa, synthetic construct
NFFYYGTTYGWYFDV

SEQ ID NO: 131 - protein, 11 aa, synthetic construct
KASEDIYNRLA

SEQ ID NO: 132 - protein, 7 aa, synthetic construct
GATSLET

SEQ ID NO: 133 - protein, 9 aa, synthetic construct
QQYWSLPWT

SEQ ID NO: 134 - protein, 5 aa, synthetic construct
NFWMN

SEQ ID NO: 135 - protein, 19 aa, synthetic construct
QIRLKSDDYATHYAESVKG

SEQ ID NO: 136 - protein, 6 aa, synthetic construct
GYYFDY

SEQ ID NO: 137 - protein, 11 aa, synthetic construct
KASENVGTYVS

SEQ ID NO: 138 - protein, 7 aa, synthetic construct
GASNRYT

SEQ ID NO: 139 - protein, 9 aa, synthetic construct
GQFYSFPCT

SEQ ID NO: 140 - protein, 5 aa, synthetic construct
NFWMQ

SEQ ID NO: 141 - protein, 19 aa, synthetic construct
QIRLKSDNYAAHYAESVKG

SEQ ID NO: 142 - protein, 8 aa, synthetic construct
GNWVGFAY

SEQ ID NO: 143 - protein, 11 aa, synthetic construct
KASQNVGTTVA

SEQ ID NO: 144 - protein, 7 aa, synthetic construct
STSNRFT

SEQ ID NO: 145 - protein, 9 aa, synthetic construct
QQYNNYPLT

SEQ ID NO: 146 - protein, 8 aa, synthetic construct
GYTFTTYG

SEQ ID NO: 147 - protein, 8 aa, synthetic construct
INTYSGVP

SEQ ID NO: 148 - protein, 11 aa, synthetic construct
ARIGDYDYGEY

SEQ ID NO: 149 - protein, 11 aa, synthetic construct
QSLLDSDGKTY

SEQ ID NO: 150 - skipped

SEQ ID NO: 151 - protein, 9 aa, synthetic construct
WQGTHFPYT

SEQ ID NO: 152 - protein, 8 aa, synthetic construct
GYTFTNYG

SEQ ID NO: 153 - protein, 8 aa, synthetic construct
INTYTGES

SEQ ID NO: 154 - protein, 14 aa, synthetic construct
ARMGDGYYDFTMDY

SEQ ID NO: 155 - protein, 5 aa, synthetic construct
SSVSY

SEQ ID NO: 156 - skipped

SEQ ID NO: 157 - protein, 9 aa, synthetic construct
QQWSSDPPT

SEQ ID NO: 158 - protein, 8 aa, synthetic construct
GYTFTGNW

SEQ ID NO: 159 - protein, 8 aa, synthetic construct
ILPGTGST

SEQ ID NO: 160 - protein, 12 aa, synthetic construct
ARWGSTVVAYDY

SEQ ID NO: 161 - protein, 6 aa, synthetic construct
KSISKY

SEQ ID NO: 162 - skipped

SEQ ID NO: 163 - protein, 9 aa, synthetic construct
QQHNEYPLT

SEQ ID NO: 164 - protein, 8 aa, synthetic construct
GYTFTSYW

SEQ ID NO: 165 - protein, 8 aa, synthetic construct
IYPGSSSP

SEQ ID NO: 166 - protein, 10 aa, synthetic construct
ARSLLYAMDY

SEQ ID NO: 167 - protein, 10 aa, synthetic construct
ESVDYDGDSY

SEQ ID NO: 168 - skipped

SEQ ID NO: 169 - protein, 9 aa, synthetic construct
LQSNEAPYT

SEQ ID NO: 170 - protein, 8 aa, synthetic construct
GYTLPGYW

SEQ ID NO: 171 - protein, 8 aa, synthetic construct
ILPGSSSA

SEQ ID NO: 172 - protein, 10 aa, synthetic construct
ASTYGTSLDY

SEQ ID NO: 173 - protein, 6 aa, synthetic construct
QSVSND

SEQ ID NO: 174 - skipped

SEQ ID NO: 175 - protein, 9 aa, synthetic construct
QQSNNWPYT

SEQ ID NO: 176 - protein, 8 aa, synthetic construct
GYTFTSYW

SEQ ID NO: 177 - protein, 8 aa, synthetic construct
IDPSDSLA

SEQ ID NO: 178 - protein, 12 aa, synthetic construct
ARDSTVVAPMDY

SEQ ID NO: 179 - protein, 6 aa, synthetic construct
KSISKY

SEQ ID NO: 180 - skipped

SEQ ID NO: 181 - protein, 9 aa, synthetic construct
QQHHEYPYT

SEQ ID NO: 182 - protein, 8 aa, synthetic construct
GYTFTSYW

SEQ ID NO: 183 - protein, 8 aa, synthetic construct
IDPSDSLA

SEQ ID NO: 184 - protein, 12 aa, synthetic construct
ARDSTVVAPMDY

SEQ ID NO: 185 - protein, 6 aa, synthetic construct
TSISKY

SEQ ID NO: 186 - skipped

SEQ ID NO: 187 - protein, 9 aa, synthetic construct
QQHHVYPYT

SEQ ID NO: 188 - protein, 8 aa, synthetic construct
GYTFTDYY

SEQ ID NO: 189 - protein, 8 aa, synthetic construct
INPYNGGT

SEQ ID NO: 190 - protein, 15 aa, synthetic construct
SRYDYDYDVEGAMDY

SEQ ID NO: 191 - protein, 6 aa, synthetic construct
QNVGTA

SEQ ID NO: 192 - skipped

SEQ ID NO: 193 - protein, 9 aa, synthetic construct
QQYSSSPYT

SEQ ID NO: 194 - protein, 8 aa, synthetic construct
GYTFTSYW

SEQ ID NO: 195 - protein, 8 aa, synthetic construct
IYPGNSDT

SEQ ID NO: 196 - protein, 11 aa, synthetic construct
TRSYDYGDLDY

SEQ ID NO: 197 - protein, 6 aa, synthetic construct
QTISDY

SEQ ID NO: 198 - skipped

SEQ ID NO: 199 - protein, 9 aa, synthetic construct
QNGHSFPLT

SEQ ID NO: 200 - protein, 8 aa, synthetic construct
GYTFTSYG

SEQ ID NO: 201 - protein, 8 aa, synthetic construct
IFPRSGNT

SEQ ID NO: 202 - protein, 13 aa, synthetic construct
ARTTVFAPYYFDY

SEQ ID NO: 203 - protein, 6 aa, synthetic construct
ENINSN

SEQ ID NO: 204 - skipped

SEQ ID NO: 205 - protein, 9 aa, synthetic construct
QHFWGLPWT

SEQ ID NO: 206 - protein, 8 aa, synthetic construct
GYTFTDYY

SEQ ID NO: 207 - protein, 8 aa, synthetic construct
ISPNYGGT

SEQ ID NO: 208 - protein, 17 aa, synthetic construct
TRSFYYYGTGYDWYFDV

SEQ ID NO: 209 - protein, 6 aa, synthetic construct
QSISNN

SEQ ID NO: 210 - skipped

SEQ ID NO: 211 - protein, 9 aa, synthetic construct
QQSNSWPWT

SEQ ID NO: 212 - protein, 8 aa, synthetic construct
GYTFTDYY

SEQ ID NO: 213 - protein, 8 aa, synthetic construct
TLPGSGSP

SEQ ID NO: 214 - protein, 15 aa, synthetic construct
ARWHYYYGSSYHFDY

SEQ ID NO: 215 - protein, 11 aa, synthetic construct
QSIVHSDGNTY

SEQ ID NO: 216 - skipped

SEQ ID NO: 217 - protein, 9 aa, synthetic construct
FQGSHVPFT

SEQ ID NO: 218 - protein, 8 aa, synthetic construct
GYAFSNYW

SEQ ID NO: 219 - protein, 8 aa, synthetic construct
INPGDGDT

SEQ ID NO: 220 - protein, 12 aa, synthetic construct
EREGRNYGDFAY

SEQ ID NO: 221 - protein, 10 aa, synthetic construct
KSVSTSGFSY

SEQ ID NO: 222 - skipped

SEQ ID NO: 223 - protein, 9 aa, synthetic construct
QHSRELPFT

SEQ ID NO: 224 - protein, 8 aa, synthetic construct
GYTFTDYY

SEQ ID NO: 225 - protein, 8 aa, synthetic construct
INPNHGDT

SEQ ID NO: 226 - protein, 17 aa, synthetic construct
ARNFFYYGTTYGWYFDV

SEQ ID NO: 227 - protein, 6 aa, synthetic construct
EDIYNR

SEQ ID NO: 228 - skipped

SEQ ID NO: 229 - protein, 9 aa, synthetic construct
QQYWSLPWT

SEQ ID NO: 230 - protein, 8 aa, synthetic construct
GITFSNFW

SEQ ID NO: 231 - protein, 10 aa, synthetic construct
IRLKSDDYAT

SEQ ID NO: 232 - protein, 8 aa, synthetic construct
TTGYYFDY

SEQ ID NO: 233 - protein, 6 aa, synthetic construct
ENVGTY

SEQ ID NO: 234 - skipped

SEQ ID NO: 235 - protein, 9 aa, synthetic construct
GQFYSFPCT

SEQ ID NO: 236 - protein, 8 aa, synthetic construct
GFAFSNFW

SEQ ID NO: 237 - protein, 10 aa, synthetic construct
IRLKSDNYAA

SEQ ID NO: 238 - protein, 10 aa, synthetic construct
TQGNWVGFAY

SEQ ID NO: 239 - protein, 6 aa, synthetic construct
QNVGTT

SEQ ID NO: 240 - skipped

SEQ ID NO: 241 - protein, 9 aa, synthetic construct
QQYNNYPLT

SEQ ID NO: 242 - protein, 7 aa, synthetic construct
GYTFTTY

SEQ ID NO: 243 - protein, 6 aa, synthetic construct
NTYSGV

SEQ ID NO: 244 - protein, 9 aa, synthetic construct
IGDYDYGEY

SEQ ID NO: 245 - protein, 16 aa, synthetic construct
KSSQSLLDSDGKTYLN

SEQ ID NO: 246 - protein, 7 aa, synthetic construct
LVSQLDS

SEQ ID NO: 247 - protein, 9 aa, synthetic construct
WQGTHFPYT

SEQ ID NO: 248 - protein, 7 aa, synthetic construct
GYTFTNY

SEQ ID NO: 249 - protein, 6 aa, synthetic construct
NTYTGE

SEQ ID NO: 250 - protein, 12 aa, synthetic construct
MGDGYYDFTMDY

SEQ ID NO: 251 - protein, 10 aa, synthetic construct
SARSSVSYMQ

SEQ ID NO: 252 - protein, 7 aa, synthetic construct
DTSKLAS

SEQ ID NO: 253 - protein, 9 aa, synthetic construct
QQWSSDPPT

SEQ ID NO: 254 - protein, 7 aa, synthetic construct
GYTFTGN

SEQ ID NO: 255 - protein, 6 aa, synthetic construct
LPGTGS

SEQ ID NO: 256 - protein, 10 aa, synthetic construct
WGSTVVAYDY

SEQ ID NO: 257 - protein, 11 aa, synthetic construct
RASKSISKYLA

SEQ ID NO: 258 - protein, 7 aa, synthetic construct
SGSTLHS

SEQ ID NO: 259 - protein, 9 aa, synthetic construct
QQHNEYPLT

SEQ ID NO: 260 - protein, 7 aa, synthetic construct
GYTFTSY

SEQ ID NO: 261 - protein, 6 aa, synthetic construct
YPGSSS

SEQ ID NO: 262 - protein, 8 aa, synthetic construct
SLLYAMDY

SEQ ID NO: 263 - protein, 15 aa, synthetic construct
RASESVDYDGDSYMN

SEQ ID NO: 264 - protein, 7 aa, synthetic construct
VASNLES

SEQ ID NO: 265 - protein, 9 aa, synthetic construct
LQSNEAPYT

SEQ ID NO: 266 - protein, 7 aa, synthetic construct
GYTLPGY

SEQ ID NO: 267 - protein, 6 aa, synthetic construct
LPGSSS

SEQ ID NO: 268 - protein, 8 aa, synthetic construct
TYGTSLDY

SEQ ID NO: 269 - protein, 11 aa, synthetic construct
RASQSVSNDLH

SEQ ID NO: 270 - protein, 7 aa, synthetic construct
YASQSIS

SEQ ID NO: 271 - protein, 9 aa, synthetic construct
QQSNNWPYT

SEQ ID NO: 272 - protein, 7 aa, synthetic construct
GYTFTSY

SEQ ID NO: 273 - protein, 6 aa, synthetic construct
DPSDSL

SEQ ID NO: 274 - protein, 10 aa, synthetic construct
DSTVVAPMDY

SEQ ID NO: 275 - protein, 11 aa, synthetic construct
RATKSISKYLA

SEQ ID NO: 276 - protein, 7 aa, synthetic construct
SGSTLQS

SEQ ID NO: 277 - protein, 9 aa, synthetic construct
QQHHEYPYT

SEQ ID NO: 278 - protein, 7 aa, synthetic construct
GYTFTSY

SEQ ID NO: 279 - protein, 6 aa, synthetic construct
DPSDSL

SEQ ID NO: 280 - protein, 10 aa, synthetic construct
DSTVVAPMDY

SEQ ID NO: 281 - protein, 11 aa, synthetic construct
RASTSISKYLA

SEQ ID NO: 282 - protein, 7 aa, synthetic construct
SGSTLQS

SEQ ID NO: 283 - protein, 9 aa, synthetic construct
QQHHVYPYT

SEQ ID NO: 284 - protein, 7 aa, synthetic construct
GYTFTDY

SEQ ID NO: 285 - protein, 6 aa, synthetic construct
NPYNGG

SEQ ID NO: 286 - protein, 13 aa, synthetic construct
YDYDYDVEGAMDY

SEQ ID NO: 287 - protein, 11 aa, synthetic construct
KASQNVGTAVA

SEQ ID NO: 288 - protein, 7 aa, synthetic construct
SASIRYT

SEQ ID NO: 289 - protein, 9 aa, synthetic construct
QQYSSSPYT

SEQ ID NO: 290 - protein, 7 aa, synthetic construct
GYTFTSY

SEQ ID NO: 291 - protein, 6 aa, synthetic construct
YPGNSD

SEQ ID NO: 292 - protein, 9 aa, synthetic construct
SYDYGDLDY

SEQ ID NO: 293 - protein, 11 aa, synthetic construct
RASQTISDYLH

SEQ ID NO: 294 - protein, 7 aa, synthetic construct
YASQSIS

SEQ ID NO: 295 - protein, 9 aa, synthetic construct
QNGHSFPLT

SEQ ID NO: 296 - protein, 7 aa, synthetic construct
GYTFTSY

SEQ ID NO: 297 - protein, 6 aa, synthetic construct
FPRSGN

SEQ ID NO: 298 - protein, 11 aa, synthetic construct
TTVFAPYYFDY

SEQ ID NO: 299 - protein, 11 aa, synthetic construct
RASENINSNLA

SEQ ID NO: 300 - protein, 7 aa, synthetic construct
AATNLAD

SEQ ID NO: 301 - protein, 9 aa, synthetic construct
QHFWGLPWT

SEQ ID NO: 302 - protein, 7 aa, synthetic construct
GYTFTDY

SEQ ID NO: 303 - protein, 6 aa, synthetic construct
SPNYGG

SEQ ID NO: 304 - protein, 15 aa, synthetic construct
SFYYYGTGYDWYFDV

SEQ ID NO: 305 - protein, 11 aa, synthetic construct
RASQSISNNLH

SEQ ID NO: 306 - protein, 7 aa, synthetic construct
YASQSIS

SEQ ID NO: 307 - protein, 9 aa, synthetic construct
QQSNSWPWT

SEQ ID NO: 308 - protein, 7 aa, synthetic construct
GYTFTDY

SEQ ID NO: 309 - protein, 6 aa, synthetic construct
LPGSGS

SEQ ID NO: 310 - protein, 13 aa, synthetic construct
WHYYYGSSYHFDY

SEQ ID NO: 311 - protein, 16 aa, synthetic construct
RSSQSIVHSDGNTYLE

SEQ ID NO: 312 - protein, 7 aa, synthetic construct
KVSNRFS

SEQ ID NO: 313 - protein, 9 aa, synthetic construct
FQGSHVPFT

SEQ ID NO: 314 - protein, 7 aa, synthetic construct
GYAFSNY

SEQ ID NO: 315 - protein, 6 aa, synthetic construct
NPGDGD

SEQ ID NO: 316 - protein, 10 aa, synthetic construct
EGRNYGDFAY

SEQ ID NO: 317 - protein, 15 aa, synthetic construct
RASKSVSTSGFSYMH

SEQ ID NO: 318 - protein, 7 aa, synthetic construct
LASNLES

SEQ ID NO: 319 - protein, 9 aa, synthetic construct
QHSRELPFT

SEQ ID NO: 320 - protein, 7 aa, synthetic construct
GYTFTDY

SEQ ID NO: 321 - protein, 6 aa, synthetic construct
NPNHGD

SEQ ID NO: 322 - protein, 15 aa, synthetic construct
NFFYYGTTYGWYFDV

SEQ ID NO: 323 - protein, 11 aa, synthetic construct
KASEDIYNRLA

SEQ ID NO: 324 - protein, 7 aa, synthetic construct
GATSLET

SEQ ID NO: 325 - protein, 9 aa, synthetic construct
QQYWSLPWT

SEQ ID NO: 326 - protein, 7 aa, synthetic construct
GITFSNF

SEQ ID NO: 327 - protein, 8 aa, synthetic construct
RLKSDDYA

SEQ ID NO: 328 - protein, 6 aa, synthetic construct
GYYFDY

SEQ ID NO: 329 - protein, 11 aa, synthetic construct
KASENVGTYVS

SEQ ID NO: 330 - protein, 7 aa, synthetic construct
GASNRYT

SEQ ID NO: 331 - protein, 9 aa, synthetic construct
GQFYSFPCT

SEQ ID NO: 332 - protein, 7 aa, synthetic construct
GFAFSNF

SEQ ID NO: 333 - protein, 8 aa, synthetic construct
RLKSDNYA

SEQ ID NO: 334 - protein, 8 aa, synthetic construct
GNWVGFAY

SEQ ID NO: 335 - protein, 11 aa, synthetic construct
KASQNVGTTVA

SEQ ID NO: 336 - protein, 7 aa, synthetic construct
STSNRFT

SEQ ID NO: 337 - protein, 9 aa, synthetic construct
QQYNNYPLT

SEQ ID NO: 338 - protein, 107 aa, synthetic construct
DIQMTQSPSSLSASVGDRVTITCRATKSISKYLAWYQQKPGKAPKLLIFSGSTLQSGVPSRFSGSGSGTDFTLTISSLQPEDFATYYCQQHHEYPYTFGGGTKVEIK

SEQ ID NO: 339 - protein, 107 aa, synthetic construct
DIVMTQSPDSLAVSLGERATINCRATKSISKYLAWYQQKPGQTNKLLIFSGSTLQSGVPDRFSGSGSGTDFTLTISSLQAEDVAVYYCQQHHEYPYTFGGGTKVEIK

SEQ ID NO: 340 - protein, 119 aa, synthetic construct
EVQLVQSGAEVKKPGASVKVSCKASGYTFTSYWMHWVRQAPGQRLEWMGVIDPSDSLANYNQEFKGRVTITVDTSASTAYMELSSLRSEDTAVYYCARDSTVVAPMDYWGQGTTVTVSS

SEQ ID NO: 341 - protein, 119 aa, synthetic construct
EVQLVQSGAEVKKPGASVKVSCKASGYTFTSYWMHWVRQAPGQRLEWMGVIDPSDSLANYNQEFKGRVTLTVDTSASTAYMELSSLRSEDTAVYYCARDSTVVAPMDYWGQGTTVTVSS

SEQ ID NO: 342 - protein, 119 aa, synthetic construct
EVQLVQSGAEVKKPGASVKVSCKASGYTFTSYWMHWVRQAPGQRLEWMGVIDPSDSLANYNQEFKGRVTLTVDTSSSTAYMELSSLRSEDTAVYYCARDSTVVAPMDYWGQGTTVTVSS

SEQ ID NO: 343 - protein, 107 aa, synthetic construct
DIVMTQSPLSLPVTPGEPASISCRASQTISDYLHWYLQKPGQSPQLLIKYASQSISGVPDRFSGSGSGSDFTLKISRVEAEDVGVYYCQQGHSFPLTFGQGTKLEIK

SEQ ID NO: 344 - protein, 107 aa, synthetic construct
DIVMTQSPLSLPVTPGEPASISCRASQTISDYLHWYLQKPGQSPRLLIKYASQSISGVPDRFSGSGSGTDFTLKISRVEAEDVGVYYCQNGHSFPLTFGQGTKLEIK

SEQ ID NO: 345 - protein, 107 aa, synthetic construct
DIVMTQSPLSLPVTPGEPASISCRASQTISDYLHWYLQKPGQSPRLLIKYASQSISGVPDRFSGSGSGTDFTLKISRVEAEDVGVYYCQQGHSFPLTFGQGTKLEIK

SEQ ID NO: 346 - protein, 107 aa, synthetic construct
DIVMTQSPLSLPVTPGEPASISCRASQTISDYLHWYLQKSHQSPQLLIKYASQSISGVPDRFSGSGSGTDFTLKISRVEAEDVGVYYCQQGHSFPLTFGQGTKLEIK

SEQ ID NO: 347 - protein, 118 aa, synthetic construct
EVQLVQSGAEVKKPGASVKVSCKASGYTFTSYWMHWVRQAPGQRLEWMGTIYPGNSDTRYNQKFKDRVTITADTSASTAYMELSSLRSEDTAVYYCTRSYDYGDLDYWGQGTTVTVSS

SEQ ID NO: 348 - protein, 9 aa, synthetic construct
QQGHSFPLT

SEQ ID NO: 349 - protein, 111 aa, synthetic construct
EIVLTQSPATLSLSPGERATLSCRASKSVSTSGFSYMHWYQQKPGQPPRLLIYLASNLESGIPARFSGSGSGTDFTLTISSLEPEDFAVYYCQHSRELPFTFGQGTKLEIK

SEQ ID NO: 350 - protein, 111 aa, synthetic construct
EIVLTQSPATLSLSPGERATLSCRASKSVSTSGFSYMHWYQQKPGQPPRLLVYLASNLESGIPARFSGSGSGTDFTLTISSLEPEDFAVYYCQHSRELPFTFGQGTKLEIK

SEQ ID NO: 351 - protein, 111 aa, synthetic construct
EIVLTQSPATLSLSPGERATLSCRASKSVSTSGFSYMHWYQQKPGQPPRLLIYLGSNLESGIPARFSGSGSGTDFTLTISSLEPEDFAVYYCQHSRELPFTFGQGTKLEIK

SEQ ID NO: 352 - protein, 111 aa, synthetic construct
EIVLTQSPATLSLSPGERATLSCRASKSVSTSGFSYMHWYQQKPGQPPRLLIYLASDLESGIPARFSGSGSGTDFTLTISSLEPEDFAVYYCQHSRELPFTFGQGTKLEIK

SEQ ID NO: 353 - protein, 111 aa, synthetic construct
EIVLTQSPATLSLSPGERATLSCRASKSVSTSGFSYMHWYQQKPGQPPRLLVYLASNLESGIPARFSGSGSGTDFTLTISSLEPEDFAVYYCQHSRELPFTFGEGTKLEIK

SEQ ID NO: 354 - protein, 111 aa, synthetic construct
EIVLTQSPATLSLSPGERATLSCRASKSVSTSGFSYMHWYQQKPGQPPRLLIYLGSNLESGIPARFSGSGSGTDFTLTISSLEPEDFAVYYCQHSRELPFTFGQGTKIEIK

SEQ ID NO: 355 - protein, 111 aa, synthetic construct
EIVLTQSPATLSLSPGERATLSCRASKSVSTSGFSYMHWYQQKPGQPPRLLIYLASDLESGIPARFSGSGSGTDFTLTISSLEPEDFAVYYCQHSRELPFTFGEGTKLEIK

SEQ ID NO: 356 - protein, 119 aa, synthetic construct
EVQLVQSGAEVKKPGSSVKVSCKASGYAFSNYWINWVRQAPGQGLEWMGQINPGDGDTIYNSKFKGRVTITADKSTSTAYMELSSLRSEDTAVYYCEREGRNYGDFAYWGQGTTVTVSS

SEQ ID NO: 357 - protein, 7 aa, synthetic construct
LGSNLES

SEQ ID NO: 358 - protein, 7 aa, synthetic construct
LASDLES

SEQ ID NO: 359 - protein, 107 aa, synthetic construct
DIQMTQSPSSLSASVGDRVTITCKASEDIYNRLAWYQQKPGKVPKLLISGATSLETGVPSRFSGSGSGTDFTLTISSLQPEDVATYYCQQYWSLPWTFGGGTKVEIK

SEQ ID NO: 360 - protein, 107 aa, synthetic construct
DIQMTQSPSSLSASVGDRVTITCKASEDIYNRLAWYQQKPGKVPKLLISGATSLETGVPSRFSGSGSGKDFTLTISSLQPEDVATYYCQQYWSLPWTFGGGTKVEIK

SEQ ID NO: 361 - protein, 107 aa, synthetic construct
DIVMTQSPDSLAVSLGERATINCKASEDIYNRLAWYQQKPGQTPKLLISGATSLETGVPDRFSGSGSGKDFTLTISSLQAEDVAVYYCQQYWSLPWTFGGGTKVEIK

SEQ ID NO: 362 - protein, 124 aa, synthetic construct
EVQLVQSGAEVKKPGASVKVSCKASGYTFTDYYMNWVRQAPGQRLEWMGDINPNHGDTGYNQKFTGRVTITVDKSASTAYMELSSLRSEDTAVYYCARNFFYYGTTYGWYFDVWGQGTTVTVSS

SEQ ID NO: 363 - protein, 124 aa, synthetic construct
EVQLVQSGAEVKKPGASVKVSCKASGYTFTDYYMNWVRQAPGQRLEWMGDINPNHGDTGYNQKFTGRVTLTVDKSASTAYMELSSLRSEDTAVYYCARNFFYYGTTYGWYFDVWGQGTTVTVSS

SEQ ID NO: 364 - protein, 107 aa, synthetic construct
NIVLTQSPATLSLSPGERATLSCKASENVGTYVSWFQQKPGQSPRLLIYGASNRYTGIPARFSGSGSGTDFTLTISSLEPEDFAVYYCGQFYSFPSTFGGGTKVEIK

SEQ ID NO: 365 - protein, 107 aa, synthetic construct
NIQMTQSPSSLSASVGDRVTITCKASENVGTYVSWYQQKPGKSPKLLIYGASNRYTGVPSRFSGSGSGTDFTLTISSLQPEDFATYYCGQFYSFPSTFGGGTKVEIK

SEQ ID NO: 366 - protein, 117 aa, synthetic construct
EVQLVESGGGLVKPGGSLRLSCAASGITFSNFWMNWVRQAPGKGLEWVGQIRLKSDDYATHYAESVKGRFTISREDSKNTVYLQMNSLKTEDTAVYYCTTGYYFDYWGQGTTVTVSS

SEQ ID NO: 367 - protein, 117 aa, synthetic construct
EVQLVESGGGLVKPGGSLRLSCAASGITFSNFWMNWVRQAPGKGLEWVGQIRLKSEDYATHYAESVKGRFTISREDSKNTVYLQMNSLKTEDTAVYYCTTGYYFDYWGQGTTVTVSS

SEQ ID NO: 368 - protein, 117 aa, synthetic construct
EVQLVESGGGLVKPGGSLRLSCVASGITFSNFWMNWVRQAPGKGLEWVGQIRLKSDDYATHYAESVKGRFTISREDSKNTVYLQMNSLKTEDTAVYYCTTGYYFDYWGQGTTVTVSS

SEQ ID NO: 369 - protein, 117 aa, synthetic construct
EVQLVESGGGLVKPGGSLRLSCAASGITFSNFWMNWVRQAPEKGLEWVGQIRLKSDDYATHYAESVKGRFTISREDSKNTVYLQMNSLKTEDTAVYYCTTGYYFDYWGQGTTVTVSS

SEQ ID NO: 370 - protein, 117 aa, synthetic construct
EVQLVESGGGLVKPGGSLRLSCAASGITFSNFWMNWVRQAPEKGLEWVGQIRLKSDQYATHYAESVKGRFTISREDSKNTVYLQMNSLKTEDTAVYYCTTGYYFDYWGQGTTVTVSS

SEQ ID NO: 371 - protein, 9 aa, synthetic construct
GQFYSFPST

SEQ ID NO: 372 - protein, 19 aa, synthetic construct
QIRLKSDQYATHYAESVKG

SEQ ID NO: 373 - protein, 19 aa, synthetic construct
QIRLKSEDYATHYAESVKG

SEQ ID NO: 374 - protein, 107 aa, synthetic construct
DIQMTQSPSSLSASVGDRVTITCKASQNVGTAVAWYQQKPGKSPKLLIFSASIRYTGVPSRFSGSGSGTDFTLTISSLQPEDFATYYCQQYSSSPYTFGGGTKVEIK

SEQ ID NO: 375 - protein, 107 aa, synthetic construct
DIVMTQSPDSLAVSLGERATINCKASQNVGTAVAWYQQKPGQSPKLLIFSASIRYTGVPDRFSGSGSGTDFTLTISSLQAEDVAVYYCQQYSSSPYTFGGGTKVEIK

SEQ ID NO: 376 - protein, 122 aa, synthetic construct
EVQLVQSGAEVKKPGASVKVSCKASGYTFTDYYMNWVRQAPGQRLEWMGIINPYNSGTSYNQKFRGRVTLTVDKSASTAYMELSSLRSEDTAVYYCSRYDYDYDVEGAMDYWGQGTTVTVSS

SEQ ID NO: 377 - protein, 122 aa, synthetic construct
EVQLVQSGAEVKKPGASVKVSCKASGYTFTDYYMNWVRRAPGQRLEWMGIINPYNGGTSYNQKFRGRVTITVDKSASTAYMELSSLRSEDTAVYYCSRYDYDYDVEGAMDYWGQGTTVTVSS

SEQ ID NO: 378 - protein, 17 aa, synthetic construct
IINPYNSGTSYNQKFRG